European Patent Application EP 4 201 949 A1, published June 28, 2023. Title: AMMONOLYSIS SOLUTION AND AMMONOLYSIS METHOD. Applicant: GENEWIZ INC., SZ. Application PCT/CN2020/125164. The sequence listing filed with the application follows.

SEQUENCE LISTING (3 sequences)

SEQ ID NO: 1 - DNA, 23 bp, Artificial sequence
  primer
cattcgtagctcggatcgtgtac

SEQ ID NO: 2 - DNA, 60 bp, Artificial sequence
  primer
gcatggcgaccttatcagtctacgtcctttgtcttcctaagaccgcttggcctccgactt

SEQ ID NO: 3 - DNA, 86 bp, Artificial sequence
  primer
gcctgcttgagcaggctgaagttggtggcacgcgtttaattaaccatatcatctagtgttgcatatgagacaaggacttttcccat